European Patent Application EP 4 144 755 A1, published March 8, 2023. Title: LABELLING COMPOSITION, METHODS AND USES THEREOF. Applicant: Universidade do Minho CENTI - CENTRO DE NANOTECNOLOGIA E MATERIAIS TÉCNICOS FUNCIONAIS E INTELIGENTES. The sequence listing filed with the application follows.

SEQUENCE LISTING (50 sequences)

SEQ ID NO: 1 - protein, 239 aa, Artificial Sequence
  rsEGFP2
MVSKGEELFTGVVPILVELDGDVNGHKFSVSGEGEGDATYGKLTLKFICTTGKLPVPWPTLVTTLAYGVLCFSRYPDHMKQHDFFKSAMPEGYVQERTIFFKDDGNYKTRAEVKFEGDTLVNRIELKGIDFKEDGNILGHKLEYNYNSHNVYIMADKQKNGIKSNFKIRHNIEDGSVQLADHYQQNTPIGDGPVLLPDNHYLSTQSKLSKDPNEKRDHMVLLEFVTAAGITLGMDELYK

SEQ ID NO: 2 - protein, 225 aa, Artificial Sequence
  Padron
MVSVIKPDMKIKLRMEGAVNGHPFAIEGVGLGKPFEGKQSMDLKVKEGGPLPFAYDILTMAFCYGNRVFAKYPENIVDYFKQSFPEGYSWERSMIYEDGGICNATNDITLDGDCYIYEIRFDGVNFPANGPVMQKRTVKWELSTEKLYVRDGVLKSDGNYALSLEGGGHYRCDFKTTYKAKKVVQLPDYHSVDHHIEIKSHDKDYSNVNLHEHAEAHSELPRQAK

SEQ ID NO: 3 - protein, 226 aa, Artificial Sequence
  NijiFP
MVNLIKEDMRVKVHMEGNVNGHAFVIEGEGKGKPYEGTQTANLTVKEGAPLPFSYDILTTAVHYGNRVFTKYPEDIPDYFKQSFPEGYSWERTMTFEDKGICTIRSDISLEGDCFFQNVRFKGTNFPPNGPVMQKKTLKWEPSTEKLHVRDGLLVGNINMALLLEGGGHYLCDSKTTYKAKKVVQLPDAHFVDHRIEILGNDSDYNKVKLYEHAVARYSPLPSQAW

SEQ ID NO: 4 - protein, 239 aa, Artificial Sequence
  Dreiklang
MVSKGEELFTGVVPILVELDGDVNGHKFSVSGEGEGDATYGKLTLKFICTTGKLPVPWPTLLTTIGYGLMCFARYPDHMKQHDFFKSAMPEGYVQERTIFFKDDGNYKTRAEVKFEGDTLVNRIELKGIDFKEDGNILGHKLEYNHDSHNVYIMADKQKNGIKVNFKIRHNIEDGSVQLADHYQQNTPIGDGPVLLPDNHYLSYQSALSKDPNEKRDHMVLLEFVTAAGITLGMDELYK

SEQ ID NO: 5 - protein, 237 aa, Artificial Sequence
  rsTagRFP
MVSKGEELIKENMHMKLYMEGTVNNHHFKCTSEGEGKPYEGTQTMRIKVVEGGPLPFAFDILATSFMYGSRTFINHTQGIPDFWKQSFPEGFTWERVTTYEDGGVLTATQDTSLQDGCLIYNVKLRGVNFPSNGPVMQKKTLGWEAATEMLYPADGGLEGRGDMALKLVGGGHLICNLKTTYRSKNPAKNLKMPGVYFVDHRLERIKEADKETYVEQHEVAVARYCDLPSKLGHKLN

SEQ ID NO: 6 - protein, 236 aa, Artificial Sequence
  mTFP0.7
MVSKGEETTMGVIKPDMKIKLKMEGNVNGHAFVIEGEGEGKPYDGTNTINLEVKEGAPLPFSYDILTNAFAYGNRAFTKYPDDIPNYFKQSFPEGYSWERTMTFEDKGIVKVKSDISMEEDSFIYEIHLKGENFPPNGPVMQKKTLKWEPSTEILYVRDGVLVGDIKHKLLLEGGGHHRVDFKTIYRAKKAVKLPDYHFVDHRIEILNHDKDYNKVTVYESAVARYSTGGMDELYK

SEQ ID NO: 7 - protein, 6 aa, Artificial Sequence
  His6
HHHHHH

SEQ ID NO: 8 - protein, 14 aa, Artificial Sequence
  CotB1p
SGRARAQRQSSRGR

SEQ ID NO: 9 - protein, 12 aa, Artificial Sequence
  Car9
DSARGFKKPGKR

SEQ ID NO: 10 - protein, 202 aa, Artificial Sequence
  CtLK-CBM3
MASTPTKGATPTNTATPTKSATATPTRPSVPTNTPTNTPANTPVSGNLKVEFYNSNPSDTTNSINPQFKVTNTGSSAIDLSKLTLRYYYTVDGQKDQTFWCDHAAIIGSNGSYNGITSNVKGTFVKMSSSTNNADTYLEISFTGGTLEPGAHVQIQGRFAKNDWSNYTQSNDYSFKSASQFVEWDQVTAYLNGVLVWGKELE

SEQ ID NO: 11 - protein, 13 aa, Artificial Sequence
  KP
GGVCGPSPPCITT

SEQ ID NO: 12 - protein, 12 aa, Artificial Sequence
  pepYN42
SYTFHWHQSWSS

SEQ ID NO: 13 - protein, 72 aa, Artificial Sequence
  BaCBM2
ATFSVTSNWGSGYNFSIVIKNSGTTPIKNWKLEFDYNGNLTQVWDSKISSKINNHYVITNAGWNGEIPPGGS

SEQ ID NO: 14 - protein, 44 aa, Artificial Sequence
  TA2(M1)
YSSCQPQGFNCKVRPYGLPTIPCCRGLTRLSYSPGSTYGRCQRH

SEQ ID NO: 15 - protein, 47 aa, Artificial Sequence
  LCI(KR-2)
AIKLVQSPNGNFAASFVLDGTKWIFKSKRYDSSKRYWVGIYEVWDRK

SEQ ID NO: 16 - protein, 248 aa, Artificial Sequence
  His6-rsEGFP2
MKHHHHHHPMVSKGEELFTGVVPILVELDGDVNGHKFSVSGEGEGDATYGKLTLKFICTTGKLPVPWPTLVTTLAYGVLCFSRYPDHMKQHDFFKSAMPEGYVQERTIFFKDDGNYKTRAEVKFEGDTLVNRIELKGIDFKEDGNILGHKLEYNYNSHNVYIMADKQKNGIKSNFKIRHNIEDGSVQLADHYQQNTPIGDGPVLLPDNHYLSTQSKLSKDPNEKRDHMVLLEFVTAAGITLGMDELYK

SEQ ID NO: 17 - protein, 264 aa, Artificial Sequence
  His6-rsEGFP2-CotB1p
MKHHHHHHPMVSKGEELFTGVVPILVELDGDVNGHKFSVSGEGEGDATYGKLTLKFICTTGKLPVPWPTLVTTLAYGVLCFSRYPDHMKQHDFFKSAMPEGYVQERTIFFKDDGNYKTRAEVKFEGDTLVNRIELKGIDFKEDGNILGHKLEYNYNSHNVYIMADKQKNGIKSNFKIRHNIEDGSVQLADHYQQNTPIGDGPVLLPDNHYLSTQSKLSKDPNEKRDHMVLLEFVTAAGITLGMDELYKHMSGRARAQRQSSRGR

SEQ ID NO: 18 - protein, 262 aa, Artificial Sequence
  His6-rsEGFP2-Car9
MKHHHHHHPMVSKGEELFTGVVPILVELDGDVNGHKFSVSGEGEGDATYGKLTLKFICTTGKLPVPWPTLVTTLAYGVLCFSRYPDHMKQHDFFKSAMPEGYVQERTIFFKDDGNYKTRAEVKFEGDTLVNRIELKGIDFKEDGNILGHKLEYNYNSHNVYIMADKQKNGIKSNFKIRHNIEDGSVQLADHYQQNTPIGDGPVLLPDNHYLSTQSKLSKDPNEKRDHMVLLEFVTAAGITLGMDELYKHMDSARGFKKPGKR

SEQ ID NO: 19 - protein, 457 aa, Artificial Sequence
  His6-rsEGFP2-CtLK-CBM3-His6
MKHHHHHHPMVSKGEELFTGVVPILVELDGDVNGHKFSVSGEGEGDATYGKLTLKFICTTGKLPVPWPTLVTTLAYGVLCFSRYPDHMKQHDFFKSAMPEGYVQERTIFFKDDGNYKTRAEVKFEGDTLVNRIELKGIDFKEDGNILGHKLEYNYNSHNVYIMADKQKNGIKSNFKIRHNIEDGSVQLADHYQQNTPIGDGPVLLPDNHYLSTQSKLSKDPNEKRDHMVLLEFVTAAGITLGMDELYKHMASTPTKGATPTNTATPTKSATATPTRPSVPTNTPTNTPANTPVSGNLKVEFYNSNPSDTTNSINPQFKVTNTGSSAIDLSKLTLRYYYTVDGQKDQTFWCDHAAIIGSNGSYNGITSNVKGTFVKMSSSTNNADTYLEISFTGGTLEPGAHVQIQGRFAKNDWSNYTQSNDYSFKSASQFVEWDQVTAYLNGVLVWGKELEHHHHHH

SEQ ID NO: 20 - protein, 261 aa, Artificial Sequence
  KP-rsEGFP2-His6
MGGVCGPSPPCITTMVSKGEELFTGVVPILVELDGDVNGHKFSVSGEGEGDATYGKLTLKFICTTGKLPVPWPTLVTTLAYGVLCFSRYPDHMKQHDFFKSAMPEGYVQERTIFFKDDGNYKTRAEVKFEGDTLVNRIELKGIDFKEDGNILGHKLEYNYNSHNVYIMADKQKNGIKSNFKIRHNIEDGSVQLADHYQQNTPIGDGPVLLPDNHYLSTQSKLSKDPNEKRDHMVLLEFVTAAGITLGMDELYKLEHHHHHH

SEQ ID NO: 21 - protein, 262 aa, Artificial Sequence
  His6-rsEGFP2-pepYN42
MKHHHHHHPMVSKGEELFTGVVPILVELDGDVNGHKFSVSGEGEGDATYGKLTLKFICTTGKLPVPWPTLVTTLAYGVLCFSRYPDHMKQHDFFKSAMPEGYVQERTIFFKDDGNYKTRAEVKFEGDTLVNRIELKGIDFKEDGNILGHKLEYNYNSHNVYIMADKQKNGIKSNFKIRHNIEDGSVQLADHYQQNTPIGDGPVLLPDNHYLSTQSKLSKDPNEKRDHMVLLEFVTAAGITLGMDELYKHMSYTFHWHQSWSS

SEQ ID NO: 22 - protein, 320 aa, Artificial Sequence
  BaCBM2-rsEGFP2-His6
MATFSVTSNWGSGYNFSIVIKNSGTTPIKNWKLEFDYNGNLTQVWDSKISSKINNHYVITNAGWNGEIPPGGSMVSKGEELFTGVVPILVELDGDVNGHKFSVSGEGEGDATYGKLTLKFICTTGKLPVPWPTLVTTLAYGVLCFSRYPDHMKQHDFFKSAMPEGYVQERTIFFKDDGNYKTRAEVKFEGDTLVNRIELKGIDFKEDGNILGHKLEYNYNSHNVYIMADKQKNGIKSNFKIRHNIEDGSVQLADHYQQNTPIGDGPVLLPDNHYLSTQSKLSKDPNEKRDHMVLLEFVTAAGITLGMDELYKLEHHHHHH

SEQ ID NO: 23 - protein, 292 aa, Artificial Sequence
  TA2(M1)-rsEGFP2-His6
MYSSCQPQGFNCKVRPYGLPTIPCCRGLTRLSYSPGSTYGRCQRHMVSKGEELFTGVVPILVELDGDVNGHKFSVSGEGEGDATYGKLTLKFICTTGKLPVPWPTLVTTLAYGVLCFSRYPDHMKQHDFFKSAMPEGYVQERTIFFKDDGNYKTRAEVKFEGDTLVNRIELKGIDFKEDGNILGHKLEYNYNSHNVYIMADKQKNGIKSNFKIRHNIEDGSVQLADHYQQNTPIGDGPVLLPDNHYLSTQSKLSKDPNEKRDHMVLLEFVTAAGITLGMDELYKLEHHHHHH

SEQ ID NO: 24 - protein, 297 aa, Artificial Sequence
  His6-rsEGFP2-LCI(KR-2)
MKHHHHHHPMVSKGEELFTGVVPILVELDGDVNGHKFSVSGEGEGDATYGKLTLKFICTTGKLPVPWPTLVTTLAYGVLCFSRYPDHMKQHDFFKSAMPEGYVQERTIFFKDDGNYKTRAEVKFEGDTLVNRIELKGIDFKEDGNILGHKLEYNYNSHNVYIMADKQKNGIKSNFKIRHNIEDGSVQLADHYQQNTPIGDGPVLLPDNHYLSTQSKLSKDPNEKRDHMVLLEFVTAAGITLGMDELYKHMAIKLVQSPNGNFAASFVLDGTKWIFKSKRYDSSKRYWVGIYEVWDRK

SEQ ID NO: 25 - protein, 234 aa, Artificial Sequence
  His6-Padron
MKHHHHHHPMVSVIKPDMKIKLRMEGAVNGHPFAIEGVGLGKPFEGKQSMDLKVKEGGPLPFAYDILTMAFCYGNRVFAKYPENIVDYFKQSFPEGYSWERSMIYEDGGICNATNDITLDGDCYIYEIRFDGVNFPANGPVMQKRTVKWELSTEKLYVRDGVLKSDGNYALSLEGGGHYRCDFKTTYKAKKVVQLPDYHSVDHHIEIKSHDKDYSNVNLHEHAEAHSELPRQAK

SEQ ID NO: 26 - protein, 248 aa, Artificial Sequence
  His6-Padron-Car9
MKHHHHHHPMVSVIKPDMKIKLRMEGAVNGHPFAIEGVGLGKPFEGKQSMDLKVKEGGPLPFAYDILTMAFCYGNRVFAKYPENIVDYFKQSFPEGYSWERSMIYEDGGICNATNDITLDGDCYIYEIRFDGVNFPANGPVMQKRTVKWELSTEKLYVRDGVLKSDGNYALSLEGGGHYRCDFKTTYKAKKVVQLPDYHSVDHHIEIKSHDKDYSNVNLHEHAEAHSELPRQAKHMDSARGFKKPGKR

SEQ ID NO: 27 - protein, 443 aa, Artificial Sequence
  His6-Padron-CtLK-CBM3-His6
MKHHHHHHPMVSVIKPDMKIKLRMEGAVNGHPFAIEGVGLGKPFEGKQSMDLKVKEGGPLPFAYDILTMAFCYGNRVFAKYPENIVDYFKQSFPEGYSWERSMIYEDGGICNATNDITLDGDCYIYEIRFDGVNFPANGPVMQKRTVKWELSTEKLYVRDGVLKSDGNYALSLEGGGHYRCDFKTTYKAKKVVQLPDYHSVDHHIEIKSHDKDYSNVNLHEHAEAHSELPRQAKHMASTPTKGATPTNTATPTKSATATPTRPSVPTNTPTNTPANTPVSGNLKVEFYNSNPSDTTNSINPQFKVTNTGSSAIDLSKLTLRYYYTVDGQKDQTFWCDHAAIIGSNGSYNGITSNVKGTFVKMSSSTNNADTYLEISFTGGTLEPGAHVQIQGRFAKNDWSNYTQSNDYSFKSASQFVEWDQVTAYLNGVLVWGKELEHHHHHH

SEQ ID NO: 28 - protein, 235 aa, Artificial Sequence
  His6-NijiFP
MKHHHHHHPMVNLIKEDMRVKVHMEGNVNGHAFVIEGEGKGKPYEGTQTANLTVKEGAPLPFSYDILTTAVHYGNRVFTKYPEDIPDYFKQSFPEGYSWERTMTFEDKGICTIRSDISLEGDCFFQNVRFKGTNFPPNGPVMQKKTLKWEPSTEKLHVRDGLLVGNINMALLLEGGGHYLCDSKTTYKAKKVVQLPDAHFVDHRIEILGNDSDYNKVKLYEHAVARYSPLPSQAW

SEQ ID NO: 29 - protein, 249 aa, Artificial Sequence
  His6-NijiFP-Car9
MKHHHHHHPMVNLIKEDMRVKVHMEGNVNGHAFVIEGEGKGKPYEGTQTANLTVKEGAPLPFSYDILTTAVHYGNRVFTKYPEDIPDYFKQSFPEGYSWERTMTFEDKGICTIRSDISLEGDCFFQNVRFKGTNFPPNGPVMQKKTLKWEPSTEKLHVRDGLLVGNINMALLLEGGGHYLCDSKTTYKAKKVVQLPDAHFVDHRIEILGNDSDYNKVKLYEHAVARYSPLPSQAWHMDSARGFKKPGKR

SEQ ID NO: 30 - protein, 444 aa, Artificial Sequence
  His6-NijiFP-CtLK-CBM3-His6
MKHHHHHHPMVNLIKEDMRVKVHMEGNVNGHAFVIEGEGKGKPYEGTQTANLTVKEGAPLPFSYDILTTAVHYGNRVFTKYPEDIPDYFKQSFPEGYSWERTMTFEDKGICTIRSDISLEGDCFFQNVRFKGTNFPPNGPVMQKKTLKWEPSTEKLHVRDGLLVGNINMALLLEGGGHYLCDSKTTYKAKKVVQLPDAHFVDHRIEILGNDSDYNKVKLYEHAVARYSPLPSQAWHMASTPTKGATPTNTATPTKSATATPTRPSVPTNTPTNTPANTPVSGNLKVEFYNSNPSDTTNSINPQFKVTNTGSSAIDLSKLTLRYYYTVDGQKDQTFWCDHAAIIGSNGSYNGITSNVKGTFVKMSSSTNNADTYLEISFTGGTLEPGAHVQIQGRFAKNDWSNYTQSNDYSFKSASQFVEWDQVTAYLNGVLVWGKELEHHHHHH

SEQ ID NO: 31 - protein, 248 aa, Artificial Sequence
  KP-NijiFP-His6
MGGVCGPSPPCITTMVNLIKEDMRVKVHMEGNVNGHAFVIEGEGKGKPYEGTQTANLTVKEGAPLPFSYDILTTAVHYGNRVFTKYPEDIPDYFKQSFPEGYSWERTMTFEDKGICTIRSDISLEGDCFFQNVRFKGTNFPPNGPVMQKKTLKWEPSTEKLHVRDGLLVGNINMALLLEGGGHYLCDSKTTYKAKKVVQLPDAHFVDHRIEILGNDSDYNKVKLYEHAVARYSPLPSQAWLEHHHHHH

SEQ ID NO: 32 - protein, 249 aa, Artificial Sequence
  His6-NijiFP-pepYN42
MKHHHHHHPMVNLIKEDMRVKVHMEGNVNGHAFVIEGEGKGKPYEGTQTANLTVKEGAPLPFSYDILTTAVHYGNRVFTKYPEDIPDYFKQSFPEGYSWERTMTFEDKGICTIRSDISLEGDCFFQNVRFKGTNFPPNGPVMQKKTLKWEPSTEKLHVRDGLLVGNINMALLLEGGGHYLCDSKTTYKAKKVVQLPDAHFVDHRIEILGNDSDYNKVKLYEHAVARYSPLPSQAWHMSYTFHWHQSWSS

SEQ ID NO: 33 - protein, 307 aa, Artificial Sequence
  BaCBM2-NijiFP-His6
MATFSVTSNWGSGYNFSIVIKNSGTTPIKNWKLEFDYNGNLTQVWDSKISSKINNHYVITNAGWNGEIPPGGSMVNLIKEDMRVKVHMEGNVNGHAFVIEGEGKGKPYEGTQTANLTVKEGAPLPFSYDILTTAVHYGNRVFTKYPEDIPDYFKQSFPEGYSWERTMTFEDKGICTIRSDISLEGDCFFQNVRFKGTNFPPNGPVMQKKTLKWEPSTEKLHVRDGLLVGNINMALLLEGGGHYLCDSKTTYKAKKVVQLPDAHFVDHRIEILGNDSDYNKVKLYEHAVARYSPLPSQAWLEHHHHHH

SEQ ID NO: 34 - protein, 279 aa, Artificial Sequence
  TA2(M1)-NijiFP-His6
MYSSCQPQGFNCKVRPYGLPTIPCCRGLTRLSYSPGSTYGRCQRHMVNLIKEDMRVKVHMEGNVNGHAFVIEGEGKGKPYEGTQTANLTVKEGAPLPFSYDILTTAVHYGNRVFTKYPEDIPDYFKQSFPEGYSWERTMTFEDKGICTIRSDISLEGDCFFQNVRFKGTNFPPNGPVMQKKTLKWEPSTEKLHVRDGLLVGNINMALLLEGGGHYLCDSKTTYKAKKVVQLPDAHFVDHRIEILGNDSDYNKVKLYEHAVARYSPLPSQAWLEHHHHHH

SEQ ID NO: 35 - protein, 284 aa, Artificial Sequence
  His6-NijiFP-LCI(KR-2)
MKHHHHHHPMVNLIKEDMRVKVHMEGNVNGHAFVIEGEGKGKPYEGTQTANLTVKEGAPLPFSYDILTTAVHYGNRVFTKYPEDIPDYFKQSFPEGYSWERTMTFEDKGICTIRSDISLEGDCFFQNVRFKGTNFPPNGPVMQKKTLKWEPSTEKLHVRDGLLVGNINMALLLEGGGHYLCDSKTTYKAKKVVQLPDAHFVDHRIEILGNDSDYNKVKLYEHAVARYSPLPSQAWHMAIKLVQSPNGNFAASFVLDGTKWIFKSKRYDSSKRYWVGIYEVWDRK

SEQ ID NO: 36 - protein, 248 aa, Artificial Sequence
  His6-Dreiklang
MKHHHHHHPMVSKGEELFTGVVPILVELDGDVNGHKFSVSGEGEGDATYGKLTLKFICTTGKLPVPWPTLLTTIGYGLMCFARYPDHMKQHDFFKSAMPEGYVQERTIFFKDDGNYKTRAEVKFEGDTLVNRIELKGIDFKEDGNILGHKLEYNHDSHNVYIMADKQKNGIKVNFKIRHNIEDGSVQLADHYQQNTPIGDGPVLLPDNHYLSYQSALSKDPNEKRDHMVLLEFVTAAGITLGMDELYK

SEQ ID NO: 37 - protein, 262 aa, Artificial Sequence
  His6-Dreiklang-Car9
MKHHHHHHPMVSKGEELFTGVVPILVELDGDVNGHKFSVSGEGEGDATYGKLTLKFICTTGKLPVPWPTLLTTIGYGLMCFARYPDHMKQHDFFKSAMPEGYVQERTIFFKDDGNYKTRAEVKFEGDTLVNRIELKGIDFKEDGNILGHKLEYNHDSHNVYIMADKQKNGIKVNFKIRHNIEDGSVQLADHYQQNTPIGDGPVLLPDNHYLSYQSALSKDPNEKRDHMVLLEFVTAAGITLGMDELYKHMDSARGFKKPGKR

SEQ ID NO: 38 - protein, 457 aa, Artificial Sequence
  His6-Dreiklang-CtLK-CBM3-His6
MKHHHHHHPMVSKGEELFTGVVPILVELDGDVNGHKFSVSGEGEGDATYGKLTLKFICTTGKLPVPWPTLLTTIGYGLMCFARYPDHMKQHDFFKSAMPEGYVQERTIFFKDDGNYKTRAEVKFEGDTLVNRIELKGIDFKEDGNILGHKLEYNHDSHNVYIMADKQKNGIKVNFKIRHNIEDGSVQLADHYQQNTPIGDGPVLLPDNHYLSYQSALSKDPNEKRDHMVLLEFVTAAGITLGMDELYKHMASTPTKGATPTNTATPTKSATATPTRPSVPTNTPTNTPANTPVSGNLKVEFYNSNPSDTTNSINPQFKVTNTGSSAIDLSKLTLRYYYTVDGQKDQTFWCDHAAIIGSNGSYNGITSNVKGTFVKMSSSTNNADTYLEISFTGGTLEPGAHVQIQGRFAKNDWSNYTQSNDYSFKSASQFVEWDQVTAYLNGVLVWGKELEHHHHHH

SEQ ID NO: 39 - protein, 261 aa, Artificial Sequence
  KP-Dreiklang-His6
MGGVCGPSPPCITTMVSKGEELFTGVVPILVELDGDVNGHKFSVSGEGEGDATYGKLTLKFICTTGKLPVPWPTLLTTIGYGLMCFARYPDHMKQHDFFKSAMPEGYVQERTIFFKDDGNYKTRAEVKFEGDTLVNRIELKGIDFKEDGNILGHKLEYNHDSHNVYIMADKQKNGIKVNFKIRHNIEDGSVQLADHYQQNTPIGDGPVLLPDNHYLSYQSALSKDPNEKRDHMVLLEFVTAAGITLGMDELYKLEHHHHHH

SEQ ID NO: 40 - protein, 262 aa, Artificial Sequence
  His6-Dreiklang-pepYN42
MKHHHHHHPMVSKGEELFTGVVPILVELDGDVNGHKFSVSGEGEGDATYGKLTLKFICTTGKLPVPWPTLLTTIGYGLMCFARYPDHMKQHDFFKSAMPEGYVQERTIFFKDDGNYKTRAEVKFEGDTLVNRIELKGIDFKEDGNILGHKLEYNHDSHNVYIMADKQKNGIKVNFKIRHNIEDGSVQLADHYQQNTPIGDGPVLLPDNHYLSYQSALSKDPNEKRDHMVLLEFVTAAGITLGMDELYKHMSYTFHWHQSWSS

SEQ ID NO: 41 - protein, 320 aa, Artificial Sequence
  BaCBM2-Dreiklang-His6
MATFSVTSNWGSGYNFSIVIKNSGTTPIKNWKLEFDYNGNLTQVWDSKISSKINNHYVITNAGWNGEIPPGGSMVSKGEELFTGVVPILVELDGDVNGHKFSVSGEGEGDATYGKLTLKFICTTGKLPVPWPTLLTTIGYGLMCFARYPDHMKQHDFFKSAMPEGYVQERTIFFKDDGNYKTRAEVKFEGDTLVNRIELKGIDFKEDGNILGHKLEYNHDSHNVYIMADKQKNGIKVNFKIRHNIEDGSVQLADHYQQNTPIGDGPVLLPDNHYLSYQSALSKDPNEKRDHMVLLEFVTAAGITLGMDELYKLEHHHHHH

SEQ ID NO: 42 - protein, 246 aa, Artificial Sequence
  His6-rsTagRFP
MKHHHHHHPMVSKGEELIKENMHMKLYMEGTVNNHHFKCTSEGEGKPYEGTQTMRIKVVEGGPLPFAFDILATSFMYGSRTFINHTQGIPDFWKQSFPEGFTWERVTTYEDGGVLTATQDTSLQDGCLIYNVKLRGVNFPSNGPVMQKKTLGWEAATEMLYPADGGLEGRGDMALKLVGGGHLICNLKTTYRSKNPAKNLKMPGVYFVDHRLERIKEADKETYVEQHEVAVARYCDLPSKLGHKLN

SEQ ID NO: 43 - protein, 260 aa, Artificial Sequence
  His6-rsTagRFP-Car9
MKHHHHHHPMVSKGEELIKENMHMKLYMEGTVNNHHFKCTSEGEGKPYEGTQTMRIKVVEGGPLPFAFDILATSFMYGSRTFINHTQGIPDFWKQSFPEGFTWERVTTYEDGGVLTATQDTSLQDGCLIYNVKLRGVNFPSNGPVMQKKTLGWEAATEMLYPADGGLEGRGDMALKLVGGGHLICNLKTTYRSKNPAKNLKMPGVYFVDHRLERIKEADKETYVEQHEVAVARYCDLPSKLGHKLNHMDSARGFKKPGKR

SEQ ID NO: 44 - protein, 457 aa, Artificial Sequence
  His6-rsTagRFP-CtLK-CBM3-His6
MKHHHHHHPMVSKGEELIKENMHMKLYMEGTVNNHHFKCTSEGEGKPYEGTQTMRIKVVEGGPLPFAFDILATSFMYGSRTFINHTQGIPDFWKQSFPEGFTWERVTTYEDGGVLTATQDTSLQDGCLIYNVKLRGVNFPSNGPVMQKKTLGWEAATEMLYPADGGLEGRGDMALKLVGGGHLICNLKTTYRSKNPAKNLKMPGVYFVDHRLERIKEADKETYVEQHEVAVARYCDLPSKLGHKLNHMHMASTPTKGATPTNTATPTKSATATPTRPSVPTNTPTNTPANTPVSGNLKVEFYNSNPSDTTNSINPQFKVTNTGSSAIDLSKLTLRYYYTVDGQKDQTFWCDHAAIIGSNGSYNGITSNVKGTFVKMSSSTNNADTYLEISFTGGTLEPGAHVQIQGRFAKNDWSNYTQSNDYSFKSASQFVEWDQVTAYLNGVLVWGKELEHHHHHH

SEQ ID NO: 45 - protein, 259 aa, Artificial Sequence
  KP-rsTagRFP-His6
MGGVCGPSPPCITTMVSKGEELIKENMHMKLYMEGTVNNHHFKCTSEGEGKPYEGTQTMRIKVVEGGPLPFAFDILATSFMYGSRTFINHTQGIPDFWKQSFPEGFTWERVTTYEDGGVLTATQDTSLQDGCLIYNVKLRGVNFPSNGPVMQKKTLGWEAATEMLYPADGGLEGRGDMALKLVGGGHLICNLKTTYRSKNPAKNLKMPGVYFVDHRLERIKEADKETYVEQHEVAVARYCDLPSKLGHKLNLEHHHHHH

SEQ ID NO: 46 - protein, 260 aa, Artificial Sequence
  His6-rsTagRFP-pepYN42
MKHHHHHHPMVSKGEELIKENMHMKLYMEGTVNNHHFKCTSEGEGKPYEGTQTMRIKVVEGGPLPFAFDILATSFMYGSRTFINHTQGIPDFWKQSFPEGFTWERVTTYEDGGVLTATQDTSLQDGCLIYNVKLRGVNFPSNGPVMQKKTLGWEAATEMLYPADGGLEGRGDMALKLVGGGHLICNLKTTYRSKNPAKNLKMPGVYFVDHRLERIKEADKETYVEQHEVAVARYCDLPSKLGHKLNHMSYTFHWHQSWSS

SEQ ID NO: 47 - protein, 318 aa, Artificial Sequence
  BaCBM2-rsTagRFP-His6
MATFSVTSNWGSGYNFSIVIKNSGTTPIKNWKLEFDYNGNLTQVWDSKISSKINNHYVITNAGWNGEIPPGGSMVSKGEELIKENMHMKLYMEGTVNNHHFKCTSEGEGKPYEGTQTMRIKVVEGGPLPFAFDILATSFMYGSRTFINHTQGIPDFWKQSFPEGFTWERVTTYEDGGVLTATQDTSLQDGCLIYNVKLRGVNFPSNGPVMQKKTLGWEAATEMLYPADGGLEGRGDMALKLVGGGHLICNLKTTYRSKNPAKNLKMPGVYFVDHRLERIKEADKETYVEQHEVAVARYCDLPSKLGHKLNLEHHHHHH

SEQ ID NO: 48 - protein, 245 aa, Artificial Sequence
  His6-mTFP0.7
MKHHHHHHPMVSKGEETTMGVIKPDMKIKLKMEGNVNGHAFVIEGEGEGKPYDGTNTINLEVKEGAPLPFSYDILTNAFAYGNRAFTKYPDDIPNYFKQSFPEGYSWERTMTFEDKGIVKVKSDISMEEDSFIYEIHLKGENFPPNGPVMQKKTLKWEPSTEILYVRDGVLVGDIKHKLLLEGGGHHRVDFKTIYRAKKAVKLPDYHFVDHRIEILNHDKDYNKVTVYESAVARYSTGGMDELYK

SEQ ID NO: 49 - protein, 259 aa, Artificial Sequence
  His6-mTFP0.7-Car9
MKHHHHHHPMVSKGEETTMGVIKPDMKIKLKMEGNVNGHAFVIEGEGEGKPYDGTNTINLEVKEGAPLPFSYDILTNAFAYGNRAFTKYPDDIPNYFKQSFPEGYSWERTMTFEDKGIVKVKSDISMEEDSFIYEIHLKGENFPPNGPVMQKKTLKWEPSTEILYVRDGVLVGDIKHKLLLEGGGHHRVDFKTIYRAKKAVKLPDYHFVDHRIEILNHDKDYNKVTVYESAVARYSTGGMDELYKHMDSARGFKKPGKR

SEQ ID NO: 50 - protein, 454 aa, Artificial Sequence
  His6-mTFP0.7-CtLK-CBM3-His6
MKHHHHHHPMVSKGEETTMGVIKPDMKIKLKMEGNVNGHAFVIEGEGEGKPYDGTNTINLEVKEGAPLPFSYDILTNAFAYGNRAFTKYPDDIPNYFKQSFPEGYSWERTMTFEDKGIVKVKSDISMEEDSFIYEIHLKGENFPPNGPVMQKKTLKWEPSTEILYVRDGVLVGDIKHKLLLEGGGHHRVDFKTIYRAKKAVKLPDYHFVDHRIEILNHDKDYNKVTVYESAVARYSTGGMDELYKHMASTPTKGATPTNTATPTKSATATPTRPSVPTNTPTNTPANTPVSGNLKVEFYNSNPSDTTNSINPQFKVTNTGSSAIDLSKLTLRYYYTVDGQKDQTFWCDHAAIIGSNGSYNGITSNVKGTFVKMSSSTNNADTYLEISFTGGTLEPGAHVQIQGRFAKNDWSNYTQSNDYSFKSASQFVEWDQVTAYLNGVLVWGKELEHHHHHH